European Patent Application EP 4 461 301 A1, published November 13, 2024. Title: A method for producing engineered platelets. Applicant: HemostOD S.A. Application EP. The sequence listing filed with the application follows.

SEQUENCE LISTING (9 sequences)

SEQ ID NO: 1 - RNA, 24 nt, Homo sapiens
  source 1..24: mol_type = other RNA
gctggtttcatatggtggtttaga

SEQ ID NO: 2 - RNA, 24 nt, Homo sapiens
  source 1..24: mol_type = other RNA
tccctgagaccctttaacctgtga

SEQ ID NO: 3 - RNA, 21 nt, synthetic construct
  source 1..21: mol_type = other RNA
acaaaacggtgtcatttgcac

SEQ ID NO: 4 - RNA, 81 nt, Homo sapiens
  source 1..81: mol_type = other RNA
cttcaggaagctggtttcatatggtggtttagatttaaatagtgattgtctagcaccatttgaaatcagtgttcttggggg

SEQ ID NO: 5 - RNA, 86 nt, Homo sapiens
  source 1..86: mol_type = other RNA
tgccagtctctaggtccctgagaccctttaacctgtgaggacatccagggtcacaggtgaggttcttgggagcctggcgtctggcc

SEQ ID NO: 6 - RNA, 60 nt, synthetic construct
  source 1..60: mol_type = other RNA
gaatctttggagtacgctggatgttttggccactgactgacatccagcgctccaaagatt

SEQ ID NO: 7 - RNA, 58 nt, synthetic construct
  source 1..58: mol_type = other RNA
gaaacctgaatctggagtacgttttggccactgactgacgtactccagattcaggttt

SEQ ID NO: 8 - RNA, 60 nt, synthetic construct
  source 1..60: mol_type = other RNA
gagtaagtcaacttcaatgtcggttttggccactgactgaccgacattggttgacttact

SEQ ID NO: 9 - RNA, 60 nt, synthetic construct
  source 1..60: mol_type = other RNA
gaaatgtactgcgcgtggagacgttttggccactgactgacgtctccacgcagtacattt